European Patent Application EP 4 130 271 A1, published February 8, 2023. Title: Modified Channelrhodopsin. Applicant: NATIONAL UNIVERSITY CORPORATION, IWATE UNIVERSITY. The sequence listing filed with the application follows.

SEQUENCE LISTING (25 sequences)

SEQ ID NO: 1 - protein, 344 aa, Artificial Sequence
  Fusion protein, mVChR1
MSRRPWLLALALAVALAAGSAGASTGSDATVPVATQDGPDYVFHRAHERMLFQTSYTLENNGSVICMPRGQCYCEGWLRSRGTSIEKTIAITLQWVVFALSVACLGWYAYQAWRATCGWEEVYVALIEMMKSIIEAFHEFDSPATLWLSSGNGVVWMRYGEWLLTCPVLLIHLSNLTGLKDDYSKRTMGLLVSDVGCIVWGATSAMCTGWTKILFFLISLSYGMYTYFHAAKVYIEAFHTVPKGICRELVRVMAWTFFVAWGMFPVLFLLGTEGFGHISPYGSAIGHSILDLIAKNMWGVLGNYLRVKIHEHILLYGDIRKKQKITIAGQEMEVETLVAEEEDR

SEQ ID NO: 2 - protein, 712 aa, Chlamydomonas reinhardtii
MSRRPWLLALALAVALAAGSAGASTGSDATVPVATQDGPDYVFHRAHERMLFQTSYTLENNGSVICIPNNGQCFCLAWLKSNGTNAEKLAANILQWITFALSALCLMFYGYQTWKSTCGWEEIYVATIEMIKFIIEYFHEFDEPAVIYSSNGNKTVWLRYAEWLLTCPVILIHLSNLTGLANDYNKRTMGLLVSDIGTIVWGTTAALSKGYVRVIFFLMGLCYGIYTFFNAAKVYIEAYHTVPKGICRDLVRYLAWLYFCSWAMFPVLFLLGPEGFGHINQFNSAIAHAILDLASKNAWSMMGHFLRVKIHEHILLYGDIRKKQKVNVAGQEMEVETMVHEEDDETQKVPTAKYANRDSFIIMRDRLKEKGFETRASLDGDPNGDAEANAAAGGKPGMEMGKMTGMGMGMGAGMGMATIDSGRVILAVPDISMVDFFREQFARLPVPYELVPALGAENTLQLVQQAQSLGGCDFVLMHPEFLRDRSPTGLLPRLKMGGQRAAAFGWAAIGPMRDLIEGSGVDGWLEGPSFGAGINQQALVALINRMQQAKKMGMMGGMGMGMGGGMGMGMGMGMGMAPSMNAGMTGGMGGASMGGAVMGMGMGMQPMQQAMPAMSPMMTQQPSMMSQPSAMSAGGAMQAMGGVMPSPAPGGRVGTNPLFGSAPSPLSSQPGISPGMATPPAATAAPAAGGSEAEMLQQLMSEINRLKNELGE

SEQ ID NO: 3 - protein, 316 aa, Chlamydomonas reinhardtii
MDYGGALSAVGRELLFVTNPVVVNGSVLVPEDQCYCAGWIESRGTNGAQTASNVLQWLAAGFSILLLMFYAYQTWKSTCGWEEIYVCAIEMVKVILEFFFEFKNPSMLYLATGHRVQWLRYAEWLLTCPVILIHLSNLTGLSNDYSRRTMGLLVSDIGTIVWGATSAMATGYVKVIFFCLGLCYGANTFFHAAKAYIEGYHTVPKGRCRQVVTGMAWLFFVSWGMFPILFILGPEGFGVLSVYGSTVGHTIIDLMSKNCWGLLGHYLRVLIHEHILIHGDIRKTTKLNIGGTEIEVETLVEDEAEAGAVNKGTGKZ

SEQ ID NO: 4 - protein, 342 aa, Artificial Sequence
  Fusion protein, p525
MSRRPWLLALALAVALAAGSAGASTGSDATVPVATQDGPDYVFHRAHERMLFQTSYTLENNGSVICMPRGQCYCEGWLRSRGTSIEKTIAITLQWVVFALSVACLGWYAYQAWRATCGWEEVYVALIEMMKSIIEAFHEFDEPAVIYSSNGNKTVWLRYAEWLLTCPVILIHLSNLTGLKDDYSKRTMGLLVSDVGCIVWGATSAMCTGWTKILFFLISLSYGMYTYFHAAKVYIEAFHTVPKGICRELVRVMAWTFFVAWGMFPVLFLLGPEGFGVLSVYGSAIGHSILDLIAKNMWGVLGNYLRVKIHEHILLYGDIRKKQKITIAGQEMEVETLVAEEE

SEQ ID NO: 5 - protein, 289 aa, Chloromonas oogama
MLGNGSAIVPIDQCFCLAWTDSLGSDTEQLVANILQWFAFGFSILILMFYAYQTWRATCGWEEVYVCCVELTKVIIEFFHEFDDPSMLYLANGHRVQWLRYAEWLLTCPVILIHLSNLTGLKDDYSKRTMRLLVSDVGTIVWGATSAMSTGYVKVIFFVLGCIYGANTFFHAAKVYIESYHVVPKGRPRTVVRIMAWLFFLSWGMFPVLFVVGPEGFDAISVYGSTIGHTIIDLMSKNCWGLLGHYLRVLIHQHIIIYGDIRKKTKINVAGEEMEVETMVDQEDEETVZ

SEQ ID NO: 6 - protein, 344 aa, Artificial Sequence
  Fusion protein, p548
MSRRPWLLALALAVALAAGSAGASTGSDATVPVATQDGPDYVFHRAHERMLFQTSYTLENNGSVICMPRGQCYCEGWLRSRGTSIEKTIAITLQWVVFALSVACLGWYAYQAWRATCGWEEVYVALIEMMKSIIEAFHEFDEPAVIYSSNGNKTVWLRYAEWLLTCPVILIHLSNLTGLKDDYSKRTMGLLVSDVGCIVWGATSAMCTGWTKILFFLISLSYGMYTYFHAAKVYIEAFHTVPKGRPRTVVRIMAWLFFLSWGMFPVLFVVGPEGFGVLSVYGSAIGHSILDLIAKNMWGVLGNYLRVKIHEHILLYGDIRKKTKINVAGEEMEVETMVDQEDEE

SEQ ID NO: 7 - protein, 311 aa, Artificial Sequence
  Fusion protein, p550
MSRRPWLLALALAVALAAGSAGASTGSNGSVICMPRGQCYCEGWLRSRGTSIEKTIAITLQWVVFALSVACLGWYAYQAWRATCGWEEVYVALIEMMKSIIEAFHEFDEPAVIYSSNGNKTVWLRYAEWLLTCPVILIHLSNLTGLKDDYSKRTMGLLVSDVGCIVWGATSAMCTGWTKILFFLISLSYGMYTYFHAAKVYIEAFHTVPKGRPRTVVRIMAWLFFLSWGMFPVLFVVGPEGFGVLSVYGSAIGHSILDLIAKNMWGVLGNYLRVKIHEHILLYGDIRKKTKINVAGEEMEVETMVDQEDEE

SEQ ID NO: 8 - protein, 344 aa, Artificial Sequence
  Fusion protein, p528
MSRRPWLLALALAVALAAGSAGASTGSDATVPVATQDGPDYVFHRAHERMLFQTSYTLENNGSVICMPRGQCYCEGWLRSRGTSIEKTIAITLQWVVFALSVACLGWYAYQAWRATCGWEEVYVALIEMMKSIIEAFHEFDEPAVIYSSNGNKTVWLRYAEWLLTCPVILIHLSNLTGLKDDYSKRTMGLLVSDVGCIVWGATSAMCTGYVKILFFLISLSYGMYTYFHAAKVYIEAFHTVPKGICRELVRVMAWTFFVAWGMFPVLFLLGPEGFGVLSVYGSAIGHSILDLIAKNMWGVLGNYLRVKIHEHILLYGDIRKKQKITIAGQEMEVETLVAEEEDR

SEQ ID NO: 9 - protein, 344 aa, Artificial Sequence
  Fusion protein, p578
MSRRPWLLALALAVALAAGSAGASTGSDATVPVATQDGPDYVFHRAHERMLFQTSYTLENNGSVICMPRGQCYCEGWLRSRGTSIEKTIAITLQWVVFALSVACLGWYAYQAWRATCGWEEVYVALIEMMKSIIEAFHEFDEPAVIYSSNGNKTVWLRYAEWLLTCPVILIGLSNLTGLKDDYSKRTMGLLVSDVGCIVWGATSAMCTGWTKILFFLISLSYGMYTYFHAAKVYIEAFHTVPKGRPRTVVRIMAWLFFLSWGMFPVLFVVGPEGFGVLSVYGSAIGHSILDLIAKNMWGVLGNYLRVKIHEHILLYGDIRKKTKINVAGEEMEVETMVDQEDEE

SEQ ID NO: 10 - protein, 344 aa, Artificial Sequence
  Fusion protein, p579
MSRRPWLLALALAVALAAGSAGASTGSDATVPVATQDGPDYVFHRAHERMLFQTSYTLENNGSVICMPRGQCYCEGWLRSRGTSIEKTIAITLQWVVFALSVACLGWYAYQAWRATCGWEEVYVALIEMMKSIIEAFHEFDEPAVIYSSNGNKTVWLRYAEWLLTCPVILIALSNLTGLKDDYSKRTMGLLVSDVGCIVWGATSAMCTGWTKILFFLISLSYGMYTYFHAAKVYIEAFHTVPKGRPRTVVRIMAWLFFLSWGMFPVLFVVGPEGFGVLSVYGSAIGHSILDLIAKNMWGVLGNYLRVKIHEHILLYGDIRKKTKINVAGEEMEVETMVDQEDEE

SEQ ID NO: 11 - protein, 344 aa, Artificial Sequence
  Fusion protein, p580
MSRRPWLLALALAVALAAGSAGASTGSDATVPVATQDGPDYVFHRAHERMLFQTSYTLENNGSVICMPRGQCYCEGWLRSRGTSIEKTIAITLQWVVFALSVACLGWYAYQAWRATCGWEEVYVALIEMMKSIIEAFHEFDEPAVIYSSNGNKTVWLRYAEWLLTCPVILIKLSNLTGLKDDYSKRTMGLLVSDVGCIVWGATSAMCTGWTKILFFLISLSYGMYTYFHAAKVYIEAFHTVPKGRPRTVVRIMAWLFFLSWGMFPVLFVVGPEGFGVLSVYGSAIGHSILDLIAKNMWGVLGNYLRVKIHEHILLYGDIRKKTKINVAGEEMEVETMVDQEDEE

SEQ ID NO: 12 - protein, 344 aa, Artificial Sequence
  Fusion protein, p581
MSRRPWLLALALAVALAAGSAGASTGSDATVPVATQDGPDYVFHRAHERMLFQTSYTLENNGSVICMPRGQCYCEGWLRSRGTSIEKTIAITLQWVVFALSVACLGWYAYQAWRATCGWEEVYVALIEMMKSIIEAFHEFDEPAVIYSSNGNKTVWLRYAEWLLTCPVILIRLSNLTGLKDDYSKRTMGLLVSDVGCIVWGATSAMCTGWTKILFFLISLSYGMYTYFHAAKVYIEAFHTVPKGRPRTVVRIMAWLFFLSWGMFPVLFVVGPEGFGVLSVYGSAIGHSILDLIAKNMWGVLGNYLRVKIHEHILLYGDIRKKTKINVAGEEMEVETMVDQEDEE

SEQ ID NO: 13 - DNA, 1026 bp, Artificial Sequence
  DNA encoding fusion protein, p525
atgtctagaaggccttggctgcttgctctggctctggctgttgcacttgctgctggatctgctggcgcctctacaggatctgatgctacagtgccagtggccacacaggacggccctgattatgtgtttcacagagcccacgagcggatgctgttccagaccagctacaccctggaaaacaacggcagcgtgatctgcatgcccagaggccagtgttactgcgaaggctggctgagaagcagaggcaccagcatcgagaaaacaatcgccatcactctgcagtgggtcgtgtttgccctgtctgtggcctgtctcggatggtacgcttaccaggcttggagagccacctgtggctgggaagaagtgtacgtcgccctgatcgagatgatgaagtccatcatcgaggccttccacgagttcgacgagcctgccgtgatctacagctccaacggcaacaagaccgtgtggctgagatatgccgagtggctgctgacctgtcctgtgatcctgatccacctgagcaacctgaccggcctgaaggacgactacagcaagagaacaatgggcctgctggtgtccgatgtgggctgtattgtgtggggagccacctctgccatgtgtaccggatggaccaagatcctgttcttcctgatcagcctgtcctacggcatgtacacctacttccacgccgccaaagtgtacattgaggcctttcacacagtgcccaagggcatctgcagagaactcgtcagagtcatggcctggacctttttcgtggcctggggaatgttccccgtgctgtttctgctgggccctgaaggctttggcgtgctgtctgtgtatggctctgccatcggccacagcatcctggacctgatcgccaagaatatgtggggcgtgctgggcaactacctgagagtgaagatccacgagcacatcctgctgtacggcgacatccggaagaagcagaagatcacaatcgccggccaagagatggaagtggaaaccctggtggccgaggaagag

SEQ ID NO: 14 - DNA, 1032 bp, Artificial Sequence
  DNA encoding fusion protein, p548
atgtctagaaggccttggctgcttgctctggctctggctgttgcacttgctgctggatctgctggcgcctctacaggatctgatgctacagtgccagtggccacacaggacggccctgattatgtgtttcacagagcccacgagcggatgctgttccagaccagctacaccctggaaaacaacggcagcgtgatctgcatgcccagaggccagtgttactgcgaaggctggctgagaagcagaggcaccagcatcgagaaaacaatcgccatcactctgcagtgggtcgtgtttgccctgtctgtggcctgtctcggatggtacgcttaccaggcttggagagccacctgtggctgggaagaagtgtacgtcgccctgatcgagatgatgaagtccatcatcgaggccttccacgagttcgacgagcctgccgtgatctacagctccaacggcaacaagaccgtgtggctgagatatgccgagtggctgctgacctgtcctgtgatcctgatccacctgagcaacctgaccggcctgaaggacgactacagcaagagaacaatgggcctgctggtgtccgatgtgggctgtattgtgtggggagccacctctgccatgtgtaccggatggaccaagatcctgttcttcctgatcagcctgtcctacggcatgtacacctacttccacgccgccaaagtgtacattgaggcctttcacacagtgcccaagggcagacctagaaccgtggtgagaatcatggcttggctgttctttctgagctggggcatgttccccgtgctgttcgtcgtgggccctgaaggctttggcgtgctgtctgtgtatggctctgccatcggccacagcatcctggacctgatcgccaagaatatgtggggcgtgctgggcaactacctgagagtgaagatccacgagcacatcctgctgtacggcgacatccggaagaagaccaagatcaacgtggccggcgaggagatggaagtggagaccatggtggaccaggaggacgaggag

SEQ ID NO: 15 - DNA, 933 bp, Artificial Sequence
  DNA encoding fusion protein, p550
atgtctagaaggccttggctgcttgctctggctctggctgttgcacttgctgctggatctgctggcgcctctacaggatctaacggcagcgtgatctgcatgcccagaggccagtgttactgcgaaggctggctgagaagcagaggcaccagcatcgagaaaacaatcgccatcactctgcagtgggtcgtgtttgccctgtctgtggcctgtctcggatggtacgcttaccaggcttggagagccacctgtggctgggaagaagtgtacgtcgccctgatcgagatgatgaagtccatcatcgaggccttccacgagttcgacgagcctgccgtgatctacagctccaacggcaacaagaccgtgtggctgagatatgccgagtggctgctgacctgtcctgtgatcctgatccacctgagcaacctgaccggcctgaaggacgactacagcaagagaacaatgggcctgctggtgtccgatgtgggctgtattgtgtggggagccacctctgccatgtgtaccggatggaccaagatcctgttcttcctgatcagcctgtcctacggcatgtacacctacttccacgccgccaaagtgtacattgaggcctttcacacagtgcccaagggcagacctagaaccgtggtgagaatcatggcttggctgttctttctgagctggggcatgttccccgtgctgttcgtggtgggccctgaaggctttggcgtgctgtctgtgtatggctctgccatcggccacagcatcctggacctgatcgccaagaatatgtggggcgtgctgggcaactacctgagagtgaagatccacgagcacatcctgctgtacggcgacatccggaagaagaccaagatcaacgtggccggcgaggagatggaagtggagaccatggtggaccaggaggacgaggag

SEQ ID NO: 16 - DNA, 1032 bp, Artificial Sequence
  DNA encoding fusion protein, p528
atgtctagaaggccttggctgcttgctctggctctggctgttgcacttgctgctggatctgctggcgcctctacaggatctgatgctacagtgccagtggccacacaggacggccctgattatgtgtttcacagagcccacgagcggatgctgttccagaccagctacaccctggaaaacaacggcagcgtgatctgcatgcccagaggccagtgttactgcgaaggctggctgagaagcagaggcaccagcatcgagaaaacaatcgccatcactctgcagtgggtcgtgtttgccctgtctgtggcctgtctcggatggtacgcttaccaggcttggagagccacctgtggctgggaagaagtgtacgtcgccctgatcgagatgatgaagtccatcatcgaggccttccacgagttcgacgagcctgccgtgatctacagctccaacggcaacaagaccgtgtggctgagatatgccgagtggctgctgacctgtcctgtgatcctgatccacctgagcaacctgaccggcctgaaggacgactacagcaagagaacaatgggcctgctggtgtccgatgtgggctgtattgtgtggggagccaccagcgccatgtgtaccggctatgtgaagatcctgttcttcctgatcagcctgtcctacggcatgtacacctacttccacgccgccaaagtgtacatcgaggccttccacacagtgcccaagggcatctgcagagaactcgtcagagtcatggcctggacctttttcgtggcctggggaatgttccccgtgctgtttctgctgggccctgaaggctttggcgtgctgtctgtgtatggctctgccatcggccacagcatcctggacctgatcgccaagaatatgtggggcgtgctgggcaactacctgagagtgaagatccacgagcacatcctgctgtacggcgacatccggaagaagcagaagatcacaatcgccggccaagagatggaagtggaaaccctggtggccgaggaagaggatcgg

SEQ ID NO: 17 - DNA, 1032 bp, Artificial Sequence
  DNA encoding fusion protein, p578
atgtctagaaggccttggctgcttgctctggctctggctgttgcacttgctgctggatctgctggcgcctctacaggatctgatgctacagtgccagtggccacacaggacggccctgattatgtgtttcacagagcccacgagcggatgctgttccagaccagctacaccctggaaaacaacggcagcgtgatctgcatgcccagaggccagtgttactgcgaaggctggctgagaagcagaggcaccagcatcgagaaaacaatcgccatcactctgcagtgggtcgtgtttgccctgtctgtggcctgtctcggatggtacgcttaccaggcttggagagccacctgtggctgggaagaagtgtacgtcgccctgatcgagatgatgaagtccatcatcgaggccttccacgagttcgacgagcctgccgtgatctacagctccaacggcaacaagaccgtgtggctgagatatgccgagtggctgctgacctgtcctgtgatcctgatcggactgagcaacctgaccggcctgaaggacgactacagcaagagaacaatgggcctgctggtgtccgatgtgggctgtattgtgtggggagccacctctgccatgtgtaccggatggaccaagatcctgttcttcctgatcagcctgtcctacggcatgtacacctacttccacgccgccaaagtgtacattgaggcctttcacacagtgcccaagggcagacctagaaccgtggtgagaatcatggcttggctgttctttctgagctggggcatgttccccgtgctgttcgtggtgggccctgaaggctttggcgtgctgtctgtgtatggctctgccatcggccacagcatcctggacctgatcgccaagaatatgtggggcgtgctgggcaactacctgagagtgaagatccacgagcacatcctgctgtacggcgacatccggaagaagaccaagatcaacgtggccggcgaggagatggaagtggagaccatggtggaccaggaggacgaggag

SEQ ID NO: 18 - DNA, 1032 bp, Artificial Sequence
  DNA encoding fusion protein, p579
atgtctagaaggccttggctgcttgctctggctctggctgttgcacttgctgctggatctgctggcgcctctacaggatctgatgctacagtgccagtggccacacaggacggccctgattatgtgtttcacagagcccacgagcggatgctgttccagaccagctacaccctggaaaacaacggcagcgtgatctgcatgcccagaggccagtgttactgcgaaggctggctgagaagcagaggcaccagcatcgagaaaacaatcgccatcactctgcagtgggtcgtgtttgccctgtctgtggcctgtctcggatggtacgcttaccaggcttggagagccacctgtggctgggaagaagtgtacgtcgccctgatcgagatgatgaagtccatcatcgaggccttccacgagttcgacgagcctgccgtgatctacagctccaacggcaacaagaccgtgtggctgagatatgccgagtggctgctgacctgtcctgtgatcctgatcgccctgagcaacctgaccggcctgaaggacgactacagcaagagaacaatgggcctgctggtgtccgatgtgggctgtattgtgtggggagccacctctgccatgtgtaccggatggaccaagatcctgttcttcctgatcagcctgtcctacggcatgtacacctacttccacgccgccaaagtgtacattgaggcctttcacacagtgcccaagggcagacctagaaccgtggtgagaatcatggcttggctgttctttctgagctggggcatgttccccgtgctgttcgtggtgggccctgaaggctttggcgtgctgtctgtgtatggctctgccatcggccacagcatcctggacctgatcgccaagaatatgtggggcgtgctgggcaactacctgagagtgaagatccacgagcacatcctgctgtacggcgacatccggaagaagaccaagatcaacgtggccggcgaggagatggaagtggagaccatggtggaccaggaggacgaggag

SEQ ID NO: 19 - DNA, 1032 bp, Artificial Sequence
  DNA encoding fusion protein, p580
atgtctagaaggccttggctgcttgctctggctctggctgttgcacttgctgctggatctgctggcgcctctacaggatctgatgctacagtgccagtggccacacaggacggccctgattatgtgtttcacagagcccacgagcggatgctgttccagaccagctacaccctggaaaacaacggcagcgtgatctgcatgcccagaggccagtgttactgcgaaggctggctgagaagcagaggcaccagcatcgagaaaacaatcgccatcactctgcagtgggtcgtgtttgccctgtctgtggcctgtctcggatggtacgcttaccaggcttggagagccacctgtggctgggaagaagtgtacgtcgccctgatcgagatgatgaagtccatcatcgaggccttccacgagttcgacgagcctgccgtgatctacagctccaacggcaacaagaccgtgtggctgagatatgccgagtggctgctgacctgtcctgtgatcctgatcaaactgagcaacctgaccggcctgaaggacgactacagcaagagaacaatgggcctgctggtgtccgatgtgggctgtattgtgtggggagccacctctgccatgtgtaccggatggaccaagatcctgttcttcctgatcagcctgtcctacggcatgtacacctacttccacgccgccaaagtgtacattgaggcctttcacacagtgcccaagggcagacctagaaccgtggtgagaatcatggcttggctgttctttctgagctggggcatgttccccgtgctgttcgtggtgggccctgaaggctttggcgtgctgtctgtgtatggctctgccatcggccacagcatcctggacctgatcgccaagaatatgtggggcgtgctgggcaactacctgagagtgaagatccacgagcacatcctgctgtacggcgacatccggaagaagaccaagatcaacgtggccggcgaggagatggaagtggagaccatggtggaccaggaggacgaggag

SEQ ID NO: 20 - DNA, 1032 bp, Artificial Sequence
  DNA encoding fusion protein, p581
atgtctagaaggccttggctgcttgctctggctctggctgttgcacttgctgctggatctgctggcgcctctacaggatctgatgctacagtgccagtggccacacaggacggccctgattatgtgtttcacagagcccacgagcggatgctgttccagaccagctacaccctggaaaacaacggcagcgtgatctgcatgcccagaggccagtgttactgcgaaggctggctgagaagcagaggcaccagcatcgagaaaacaatcgccatcactctgcagtgggtcgtgtttgccctgtctgtggcctgtctcggatggtacgcttaccaggcttggagagccacctgtggctgggaagaagtgtacgtcgccctgatcgagatgatgaagtccatcatcgaggccttccacgagttcgacgagcctgccgtgatctacagctccaacggcaacaagaccgtgtggctgagatatgccgagtggctgctgacctgtcctgtgatcctgatccgcctgagcaacctgaccggcctgaaggacgactacagcaagagaacaatgggcctgctggtgtccgatgtgggctgtattgtgtggggagccacctctgccatgtgtaccggatggaccaagatcctgttcttcctgatcagcctgtcctacggcatgtacacctacttccacgccgccaaagtgtacattgaggcctttcacacagtgcccaagggcagacctagaaccgtggtgagaatcatggcttggctgttctttctgagctggggcatgttccccgtgctgttcgtggtgggccctgaaggctttggcgtgctgtctgtgtatggctctgccatcggccacagcatcctggacctgatcgccaagaatatgtggggcgtgctgggcaactacctgagagtgaagatccacgagcacatcctgctgtacggcgacatccggaagaagaccaagatcaacgtggccggcgaggagatggaagtggagaccatggtggaccaggaggacgaggag

SEQ ID NO: 21 - DNA, 26 bp, Artificial Sequence
  172G forward primer
ggactgagcaacctgaccggcctgaa

SEQ ID NO: 22 - DNA, 24 bp, Artificial Sequence
  Reverse primer
gatcaggatcacaggacaggtcag

SEQ ID NO: 23 - DNA, 26 bp, Artificial Sequence
  172A forward primer
gccctgagcaacctgaccggcctgaa

SEQ ID NO: 24 - DNA, 26 bp, Artificial Sequence
  172K forward primer
aaactgagcaacctgaccggcctgaa

SEQ ID NO: 25 - DNA, 26 bp, Artificial Sequence
  172R forward primer
cgcctgagcaacctgaccggcctgaa